European Patent Application EP 4 421 089 A1, published August 28, 2024. Title: Purification Method for fusion proteins with IgG Fc domain. Applicant: Alteogen, Inc. The sequence listing filed with the application follows.

SEQUENCE LISTING (4 sequences)

SEQ ID NO: 1 - protein, 222 aa, synthetic construct
TCPPCPAPELLGGPSVFLFPPKPKDTLMISRTPEVTCVVVDVSHEDPEVKFNWYVDGVEVHNAKTKPREEQYNSTYRVVSVLTVLHQDWLNGKEYKCKVSNKALPAPIEKTISKAKGQPREPQVYTLPPSRDELTKNQVSLTCLVKGFYPSDIAVEWESNGQPENNYKTTPPVLDSDGSFFLYSKLTVDKSRWQQGNVFSCSVMHEALHNHYTQKSLSLSPG

SEQ ID NO: 2 - protein, 224 aa, synthetic construct
THTCPPCPAPELLGGPSVFLFPPKPKDTLMISRTPEVTCVVVDVSHEDPEVKFNWYVDGVEVHNAKTKPREEQYNSTYRVVSVLTVLHQDWLNGKEYKCKVSNKALPAPIEKTISKAKGQPREPQVYTLPPSRDELTKNQVSLTCLVKGFYPSDIAVEWESNGQPENNYKTTPPVLDSDGSFFLYSKLTVDKSRWQQGNVFSCSVMHEALHNHYTQKSLSLSPG

SEQ ID NO: 3 - protein, 229 aa, synthetic construct
HEKDKTHTCPPCPAPELLGGPSVFLFPPKPKDTLMISRTPEVTCVVVDVSHEDPEVKFNWYVDGVEVHNAKTKPREEQYNSTYRVVSVLTVLHQDWLNGKEYKCKVSNKALPAPIEKTISKAKGQPREPQVYTLPPSRDELTKNQVSLTCLVKGFYPSDIAVEWESNGQPENNYKTTPPVLDSDGSFFLYSKLTVDKSRWQQGNVFSCSVMHEALHNHYTQKSLSLSPG

SEQ ID NO: 4 - protein, 230 aa, synthetic construct
VHEKDKTHTCPPCPAPELLGGPSVFLFPPKPKDTLMISRTPEVTCVVVDVSHEDPEVKFNWYVDGVEVHNAKTKPREEQYNSTYRVVSVLTVLHQDWLNGKEYKCKVSNKALPAPIEKTISKAKGQPREPQVYTLPPSRDELTKNQVSLTCLVKGFYPSDIAVEWESNGQPENNYKTTPPVLDSDGSFFLYSKLTVDKSRWQQGNVFSCSVMHEALHNHYTQKSLSLSPG